European Patent Application EP 4 279 502 A1, published November 22, 2023. Title: Compound or salt thereof or antibody obtained thereby. Applicant: Ajinomoto Co., Inc. The sequence listing filed with the application follows.

SEQUENCE LISTING (9 sequences)

SEQ ID NO: 1 - protein, 449 aa, Artificial Sequence
  Amino acid sequence of heavy chain in trastuzumab
EVQLVESGGGLVQPGGSLRLSCAASGFNIKDTYIHWVRQAPGKGLEWVARIYPTNGYTRYADSVKGRFTISADTSKNTAYLQMNSLRAEDTAVYYCSRWGGDGFYAMDYWGQGTLVTVSSASTKGPSVFPLAPSSKSTSGGTAALGCLVKDYFPEPVTVSWNSGALTSGVHTFPAVLQSSGLYSLSSVVTVPSSSLGTQTYICNVNHKPSNTKVDKKVEPKSCDKTHTCPPCPAPELLGGPSVFLFPPKPKDTLMISRTPEVTCVVVDVSHEDPEVKFNWYVDGVEVHNAKTKPREEQYDSTYRVVSVLTVLHQDWLNGKEYKCKVSNKALPAPIEKTISKAKGQPREPQVYTLPPSREEMTKNQVSLTCLVKGFYPSDIAVEWESNGQPENNYKTTPPVLDSDGSFFLYSKLTVDKSRWQQGNVFSCSVMHEALHNHYTQKSLSLSPG

SEQ ID NO: 2 - protein, 214 aa, Artificial Sequence
  Amino acid sequence of light chain in trastuzumab
DIQMTQSPSSLSASVGDRVTITCRASQDVNTAVAWYQQKPGKAPKLLIYSASFLYSGVPSRFSGSRSGTDFTLTISSLQPEDFATYYCQQHYTTPPTFGQGTKVEIKRTVAAPSVFIFPPSDEQLKSGTASVVCLLNNFYPREAKVQWKVDNALQSGNSQESVTEQDSKDSTYSLSSTLTLSKADYEKHKVYACEVTHQGLSSPVTKSFNRGEC

SEQ ID NO: 3 - protein, 18 aa, Artificial Sequence
  Amino acid sequence of peptide fragment  obtained by cleaving trastuzumab with trypsin
FNWYVDGVEVHNAKTKPR

SEQ ID NO: 4 - protein, 34 aa, Artificial Sequence
  Affinity peptide capable of binding to CH2 domain of immunoglobulin unit
FNMQCQRRFYEALHDPNLNEEQRNARIRSIKDDC

SEQ ID NO: 5 - protein, 34 aa, Artificial Sequence
  Affinity peptide capable of binding to CH2 domain of immunoglobulin unit
FNMQCQRRFYEALHDPNLNEEQRNARIRSIKEDC

SEQ ID NO: 6 - protein, 34 aa, Artificial Sequence
  Affinity peptide capable of binding to CH2 domain of immunoglobulin unit
FNMQCQRRFYEALHDPNLNEEQRNARIRSIKEEC

SEQ ID NO: 7 - protein, 33 aa, Artificial Sequence
  Affinity peptide capable of binding to CH2 domain of immunoglobulin unit
NMQCQRRFYEALHDPNLNEEQRNARIRSIKEEC

SEQ ID NO: 8 - protein, 32 aa, Artificial Sequence
  Affinity peptide capable of binding to CH2 domain of immunoglobulin unit
MQCQRRFYEALHDPNLNEEQRNARIRSIKEEC

SEQ ID NO: 9 - protein, 31 aa, Artificial Sequence
  Affinity peptide capable of binding to CH2 domain of immunoglobulin unit
QCQRRFYEALHDPNLNEEQRNARIRSIKEEC